European Patent Application EP 4 728 867 A1, published April 22, 2026. Title: BACTERIOPHAGE COMPOSITION AGAINST BACTERIAL CANKER IN SOLANACEAE. Applicant: De Ceuster Meststoffen N.V. The sequence listing filed with the application follows.

SEQUENCE LISTING (2 sequences)

SEQ ID NO: 1 - DNA, 15103 bp, unidentified
  source 1..15103: mol_type = genomic DNA
atggactcgacgcggaatcagtgcccgaagccgctgttcgacagcgcgtatgacaacgccgacgagtgggctgacgagttccgcgccgggtgggccgcgatggcgacgctcgaccgcgcgaccggcgagccgatcctgccgaagccgcagagctggctcatcgccgacgcgatgaacgctcacgacctcgacaccgggatgcccctgcactcgaccctcggcatatgcgtgccgcgtcgtgcagccaagacgacgtcgatcctcgccgtcgccctcggccggtgcatcacgcgccccggctacgtcgtgctgttcacggcccagtccggcacgaaggcgtccgcgcgcttcctggacctcgcccgtgcgctcgaccgggtgaacagcaacgacgagcagcgcggcttccgcatccttcgaggggccggaaatcagctcatcgagttcgccaacgggtcgctcttcctcgtcgtgcccccgaagggcgacagcttccgcggcgacgcgggcgacctgatcgtgctcgacgaggcgcaggcgcacgacccggtcgacagtgaggacctgatcggcgccatcctgcccgtgatggacacgcggccgggcgcgcagctcgtcgtcgccgggaccgccggggagcatcggtccggcctgttctgggacacgctcgaagagggccggaaggccgtgctcggcaccggcatcgtcgagttcgcggcgcacccggatacgcctatccacatcgagggcgagccggtcgagggcaccgtcgcggacccggctgtctgggagcgcacgcaccccggcatcgggacgctgacgaccgtcgagaccgtcgccatccggtacgcgaagctggggctcccccagttcatgcgcgagtacctggggatatggccggaggacttcacgcagtccgccatcccggccgacaagtggcgcgacggagccgagcctttcagcccgaagcccgacgacttcgcgctcgcgttcgacgtctcgccggacggcagctcggccgccatcgtcgccgcgtggcgcaaccggtcgggcgtcgccttcgtcgaggtcgtccggcacgagcccggcagctcatggctcgtgcccgccctcgtcgacctgtccaagcggtaccgggtgacggtcgggcacgacaccatcggcgcggccttcgtcgaggccgaagccctcggccgggagcgcccgaagccgaggctccgccctatgatgatgcgcgacgtcggcgcaggctgcgccgccatcatgaaggaaatccagtccggcaacctgattcacttcgatcagcccgggctcaacaccgcagccctgaacgtctcgaagcggcccctcggcgaaaacgcatgggcctggggccggaaggcgtcgaaggccgatatcgggccgctcatcgccgcgacgcacgcgctgcgcgtctacgattcaacacaatccacgccgtctctcggcgtgatatcagctaagggaatgggactgtaggcatatgggaatcttcgacagcgtcggccgagcgctcggcttccgatccgggacgtcgcagatgggcgtccggtcggcattcagtcagggcggcctcgagaaattggtctactccgacctgttcggcgtcgccccggcgatcatcagccgcgaggagggcctgtcgctgcccgccgtggcgaaggcccgggccgtcctcacggggcagatcagccggtggccgctcgtcgtgctcgacgtgaacggtccggccgccgcgcagccggaatggctacagcgcacgacgggcgaggtcagccccttccatcggatgctactgacggtcgacgacctgctgttcatgggctggtcgctgtgggccgtcgagcgcgacgcgccgagcgtggagggcgcgatcctcgaagccgagcgcctggcacccgaccgctggcagatgctcgcggacggcgagctgcgcgtcgacgacaagcccgtggacgagtgggccgtgatcctgattcccggcccgcagccgggcctgctcgacctcgcctcgcggacgctccgcggaggcgtcgagctcgaacgctcatgggtcaagcgcgccaagaatccgatcccggccatcaacctgcaagaggtcgaggagggccgcacgacgcgggacgaggcggtcgagaccgtgaaggcgtgggctcaggcgcgcgacgacgagaacggcgcaatcgcgttcacgcccgcatcgctgaaggtcgaagcgctcggcgaaatcaacgcgcagctcttcgtcgagggccgtaacttcttccggctcgacgtcgccgcgatgaccaacatccccggcgcgatcctcgacgcctcgcaggccgaggcgtccctgacgtacacgacgcaggagggcaaccgctccgagttcgcaacgatgacgctcccgtactggatgggtgccatcgagggccgcctgtcgcaagacgatgtcgtgccgcgggggcagcgtgtacgcttcgacctgaccgacgcctacgcggcgacgaccgcccccaccgggccgaccacgagggactgaccacatgaccaccgttcaattcgaagggcagacactccacgcgagcgtcgccgaccgactcgtctccgggatgctcctcccgttcggcgtgctcggcaacaccaacctcggccgcttcacggtcgacgccgggacgttcacgtacccgaccgacgtcaccgtgctcaacgccaacgaaggccacctgccgcacgagccccgagcccgcttcgcgtccctcaccgagacccccgccggtctgctcgccgccttccgcgtcgcggacggccccgagggcgacacgctgctcgcccgcctcgccgacccgaacgatgccgaggccccgcgcagcctgtccgtcgaggttcacgacgtcgtcgtgaaggcgggcaaggccatcaagggccgcatcttcggcgcggccttcgtcaagcgcggagccttcccgggcgctacgctcatggcggccgacttcggcgacgagcagccggccgaggtcgtcgtccccgacgccgtcgtgaccgaggccaccgccgacgtcgtgcagctcgacgtcgtcaccgtccccgagcgcgtcaccgtcaccccccggggtgagggtgccgagcccgtcaacttcacccccgagaacaccaaccccaacccgtccgaggaggacactttgaacgctgccgcaccccagaccttcggcatccgccggaccccgaccgcgcagacgaccggcgacggccgttcgctccgcgacatctgcaccctgctcgccatgagcgcgaccgactccggcgcggcgcgcgacctgcacgccgagttcgccgcgtccggcgacctcttcgccgccctcgtcgacgtgaagcacgacggcaccggcacgaccggcgaggccacccgcctgccgcagtgggtcggcgagctgtggaacgggcgtctcttcgagcgccgcatcgttccgctgttcgcgcacgcggacctgaccgccatcgacatcaagggatgggaatgggacgtgaagcccgtgatggccgagtggaccggcaacaaggccgccgtcccgtccgccgcgatcagcacgaagcccggcaccggcaaggccaagcgctacgccggggcgcacgacatcgcccgcgagttccgcgacttcccgaaccccgagttctgggagggatacttccgcgcgatgaccgagagctacgcgcgcctcaccgacgccgcgaccctcgtcgacgcgctcagctactcgaagcccgtcgtgcagggtgccatcccgtccggcatcgcgcccggcatggcccgcatcgtggacggcgcgctggccgtcctcgacgagggcctgccgaccttcgccgtcgtcaacaaggccgactaccgggacatcctgctcacccgcaacgatgacaccctggcctacctcaacgcggccctcggcctcgaagagggcaccgtgtcgagcttcaaggtcgtcccccacgggtcgatcccggcgaacaagacgctcgtcggcatcacgtcggccctgaccgtccacgagctgcccggctcgccgatccgcaccgaggcgctcgaccaggtcaagggcggcgtcgacgaggcgctgttcggctacgcgggcacgatgcgccacgacaccgacgccctggccctcgtcggcccggcggcctagctcgaccccgaggggcgggcgtcaggcatcccctgacgcccgcccctcccctcatccaccatccgcacgacctcacaggaaggccccatcatggcggtcccttacacccgcaaaacgtggtacaactcccccgacacccgcacgccgatcagcggcgacgggctcaacgacttcgagcgccgcgtcgcggcaggcttcgccgccgtccccgagggcggcaccggcggctccggcacgatgtcgcgcgacgcggtcggcgtggccgccctcttcgcgtccctcgacatgaaggatccccgcccgctgtccgtctacatctgctccgactcgaccggcgtcccggccgcagcgtggcaggaggccgcatggaaggccctgctcgcctcgcactaccccgagcgccaggccctcgtgcgccgcgccacgaccggcggcacgctcgcctcggccgtgcagtggcaggccgggacctccggcggcggcggcaccggcacccccgtccgcgagaagatcaccgtcctacaggacaccttcgccgggcagccgggcgagctggtcggcacgacgccgaccggtccggccggtggcaactggtcgaccatcacgggcggcacggggcagttcacccgcgccacgaccgcgtcgagcttcgtcgagtcgacgtccggccgcgtggccgacatcggcaagagcgactacgtcctgtacgccgcgagcgacgcgaccgccgagtccgacctcgacgtgacgctgcgcatctcgaccaacagcgcgtcggcagtcacgacgcgcctgttccccatccgcaaggccaacaacgacgggacccggatcgaggtcgtcgcctcgtccgccgggacgtcggtcacggtctacgcccgcacgtcggccgtcacccggaccctcggcagcatcacgggcacgccgatcccgctgaacaccgtgaacaacttcgtgcggatcaagcacgccatcgtcgccgacgcgagcggcggcacgggcgtcctgacggtcacggtcgggtcgcagaccgcgagcttcccgctgacggccgccgacatgaccgcctacagctccggcgaccgcttcgagttcgcgtcgacggacccgacgttccgcatggcgaccgtcacggcgtcgagctaccggaccacgacgtcgggcggcggcacgggcgggctcccgcccatcacgatctacaacctgtcggcgtccggtcagacggcgcagtggcagcaggaccgcatcggggcgctgttcccggcccggcccgacctcgtgatgaacaaccacggcatgaactacgaagccgacgcccccgacgtgtacctcgccaagctcgcggccttcgagtcggccgtcgccgccgcgttcgacgacgccgtgcctcactggtacgtctcgcccaacacccgcgtaccggcgtccggcgtgccctccgaccgcgtgccctccgaccgcgtgccctcgcaccgtgcccgcacggtcgcgctgcgctcgtggacggcgagccggggcacgccctactccggcgtctatgagcgcttcgcgcagcgctccgacgacggcgcggggatcctgctcgacgacaagcaccccgacgcgaccggcaacgccctggggaccggcgtcgtgcgcgccgacctcgcggcctgctcgaagcgggtcccggcgtgatcgaggccacgagcgccgcgaggtcgtcattctggatcggcgacctgccgccttcgcccctcgtcgtcaccatcacggccgacgagggcgaggccgacgccttcgagcggttcacggtcgcggccctgctcgtcagcccgaccggcgtcaggacggccctgacggccgctccggcgggtgacgacgtcgcggtctcgtggccgaccatgtcgccgttcacggaggccggtatctacgccctgacgctcaccctgtcgagcgtcgtcccggtcgcgccggtcacgctgcgcgcgaccccgctgcgcttcgtcgtgcagcgcgaggacgagtggatcaccgtggaccaggcgcgcgaggactggccggacgcgccctcgtcggacgtccggctctacgccctcctctcggccgcccgggagcagtgcgaggcgtacgcgccccgcctgctcccgggggtccgggtcccggcccgctaccgggaagcgcagctcatgcagacggccgccctgtggcaggcgaataagaccggcgacggcgacgtgattggcgccgatggcacgacggtccgcgtctatccgatgggctggaacgtcaaggccgtcctccggccgccgagcggggggcacaacgtcgcatgaacgccgcgaagctcaacacccctgcccggcagctagaagcgtttctccgggccgatgagcggttcgcccgctatcggctcatcccgaacagcatcgcccggaccggcaacctcgaccggccgacgctgcgcatcgtgcatagcgaccggcagccctcgcggttcgccgccggtttctggctcgacgagctgcgcgtcgtcctctacgtgcccggcatcgccgagtcgaccgaggacgacctagactccgagttggtcaccctcggcgacctgctcgaagatacgccgagcatcaacttcgtccgcgccgagcggacgacgaccgacgagttcaacacctggacttgcaccgtggaaatacacactcagaaagtgagctagctcatggcaaccatcgacccgaagcccttcgtcctcaaagacatgctcatggcgaacccgaccgacagcttcgagaagcaggtctcggccgtcatcctgacgcccaccgtcagcgtgcagtcgtggcagggcggcaccccggcggcgacgtacagcgacacgacgccctcgacgtggacgtgccagatcgactacgcgcaggactgggagacgaccggcagcctctcgcagtacctcttcgacaacgaaggcaagcagatcacctggaagttcacgccgatcaagggtcgcggcaagacctggaccgtcgtggcgaccatcgtccccggcaccatcggcggcagcgtctcggccttcgccacggcgtcggtcacgatgcccgtcacgggcaagccctccgcggccgcggcggcggcgtagcgtgccggtcgacgtccggcagtcaccggagctacaggcgatcatcttcgccatcaaggctgccaacgccgacctccgcaagatcctgctccgcgagtcccgccgcgtgctccgcgcggcgtgggccgaggagctgaaccaacgggcgagcacgccgctagagcagcgcgtgctcgcccgcggttcgtccgtccgggtcgggcaagccctgtccgtccgggcggcctactcgaagcggaagctcgaaggcggcctgaccccggccgaggacttcgcatcggtcgagctgggagccaagtggaagaaggccaccattcgcgcgacgtcgtcgaagggtaaggcattcacgtataccaagacgatcaataagcaattcaagcctcgacgtcgaaagggatatgtcgtattcccggcggctaagaaggtcggaaatagaatgaccgccctttgggtgcagacaatcgtaaagacataccgtgatgcggtcgaagggaagatgaactaatggccggtggcggaattgaaatcccgttcacttcgaatacgcgcgacctgctgcgcggaacgaaggacgtacagggtggactagaggacgtgcaggacagcctcgacgacctcgtgaaagcgaccgataaggacgctatctcgaagagcatggggaaggaggcgaaagaggtcgagcgcgagaccgagcggatggagaagagcttcgaggagctgtccgacacgcagaagcgcgagaccaagggcctcggcgacggcatcggcgagaacgtcaagcgcgggaccgacgaggccggggaagggctcgacgagttcaaagacgaagccaactcgaccgcgaaggagaccgcggcgagcttcgacggctcggccgacagcatcgtcggatcctttcaggaagtgctcgccaacgccttcgcaggcttcggccccgcgggagcagcggccgggctcgccctcgccatcgggctcggcaccgcggtacaggccgggcaggacgccgccgacgcgatcaacgaagccaagacccggagcggggaactagccctcgaaatcatcgacgccgggggcgacatcgcgcaggtggacatcggggcgaagatccgcgattggggcatcgcgatcgacgacaaccgcgagttctgggagctgtggcagggcagcgcgacgaacaacatggacaaggccatgcggtacgcgaagctgaccgggtcgagcttcgaggccatgttccgcggcctgtccggctatgacgccgacgccgcctccgacgtgctcgacgacgtcgccggacagatcgacgacctagagcgcaagatccgcgacgcccgcagctccggcaacgtctttgcgggcgtgcaggacgaggacgggcaggcgctcgactccctccgcggcgtccggaaagagctgaccaacgtccgcgacgagacgaaggatgccgccgccgcggcgaagctcatggaggacgcgacccgggccgagtccgacgcggccgaggcggcgaccgaggcgcagcaggcgcgagccgacgcggtctcgtcgctacagtccggcatcgacgacgcggtcggggcctatggcgagttcatggggaaagagggcgaggtcgccgacccgtccgcctacatcgccgggatccgcgaccgcatcgcggcgacgggtgacttcaatgggaacgtgcagcgcctcgcgtccgagttcggcctgtcgcaggcaggcatccagtcgatcatcgaccaggggatcgacttcgcgccgatgttgcagagcatcctcgacagcggcctcgcgcccgagtacgtcgcgcagatcgaggcggccctgaacggggggcagaacgccatcgacgggacgccccttagctcgaccgtcgacgtcgacgccgacacgtcgcaggccgagcgcgacgtgaagggcgtcgagtccaagccccggaagaccgacgtcgacgtgaaggcgcagacgaaggccgcgagccgggacatcgacgccgtggcgaaggcgaagcggacggcgaccatcgacgtccgggccgacaccggatccgcccgccgcgccatcgaccggctcggcgacgagcggaccgctacgattcgagcggtcgcatcgaccggcgcggccgaccgcgcgctcgacaacctcgcatcgcagtatcgaaccgcgacgatccacgcacgggtcgtcgaccgcaacggaaagcaggtcagctagtgcccgcaacgatcacggccccggacggcgcgcagctccgccccgtgctgatcctcgctcacgagacaagccgagacctcggcacgcgagcgcacaccgtgctcggctcggccgtccccgagttcacctactcgcagccgggcacgcgcacgggcgagctgcgcctgttctgggacagctacgcccccgtagccgccgcgcagcgcgccctcgtcaagcccggcctcttcgccatgcgcaaccccgaagagcccgagtggaacatgaccttcgccgcggtcgggtcgatgaacgtcgagcggctgggagaggacggcatccgcgtgttcggcctgtcggtcggcttcgtcgaagccttcgaggcagtgaacgccttcgccctctacccgtccccggacctctacccgtccgacgacctgtacccggcggcctgacgtgtactcccgtcacggcgcgaccgtcgagctggtcgtccccggatccgtcccggtccgcgtgctgtccggcacgctcacgatggacgagggttggtcgccgtacgcgcaggccgacctcgtcgccgtgctcgcgccgcaggcgaacaccatcgacccccgaaccgccgacgtcagggcgatcctgacgctgtctgtcgagtacggcgacagcgacaccctcgccgacctcacggcacgctaccccggcacgctcgccgacgtcacccggaagctcggcgggatgaccctcggcgagctgacccggtcgagctatgtccccttcgtgcccggcgagtaccgggaggcggtcgtgcggacgttcgacctcggcgtccgcgagattgagcgcgacctgacggcgggcgagatgacgctgcgcctcgcgtccgacgaagccctcgtgcaggacgatgcgctgatcgacggcgcgccgtacgcgatgaacgtgcagtcgctccggcaggccgtcaacaccgtcctcgcccggaagggcatggcgctgtccaccgacgaacaggacgactaccggctcgaaccggcgtcgacgacgtgggatcccgggcaatcgggatgggactttctcgagcccctggtgcagccgtccggccttcgtctttggtgcgacgaggatcggcggtggcacctgtcccgctccgagaccgccgagcgggccgacatcgtcgtggcggcgggcgtgaacatgaccggcgcgcaggacaagctcagccgggatgacgactggtactccgccgtcatcatcacgtacgaatggcgcgagcaggtcggcgaggacaccgtcgaccgcatcgcctatgacgccgcccgcctgcccggaccggcccgcgtgctcgccctcagctaccggacggcctaccccggccccggagctgcgcaggccctcctcacccgagcacggtcccgcggccgggcgatgcccgtcacggcgatcagcgactacgcggcgaccccggggaacaccattcggatccaagccccgcagacggccgcgcagcgcgccatcctcgcgtcggtacgattcgacctgttcgaccatgaaatgcaagtcacgagccgagacctacaggagacgacctaatgcccatcgacccggataccggcgtacacatctacaccgagcaggagagcgtcggccgctggtccgacatgctgaacaaagggcagcgggcgatgcagaccgtcgtccggcagctctcgaagggccgcctcgtggcgacgcacgatgcgccgtggcagcccgaccggcggctcatcacgggcgacctcgtccgcctctacgagtggtacgtgccggatcccggcttcccgtacaagatcagcgtcgaggtcacctgtgagatgggcggcctcaaccgcgacacccggtatgacctgtcggtcggatacggcgggtcgccgggcggatcctacgatcagcagatcggcttccatgtcaacctggcaggcgaggccaccttccagtcctacagcgggcagccgatcccgaccgtgcttaccggcccgacccgcatcgccgtcatggccggtgcggtctacgggccgtcaccccggcagggcgtgctcgcgcagtacaacgcccgccttcgcgtcgcggtctacagcgcctagtctgtagatcatccacaggccggcccgccgagctcggcgggccggcctagccaacacctacaaaggaagcatcatcatgaccgtctacgtcagccccgcccctcacgccgagcgcatcacggacaactacgccgcgcacgtcaagcgccgcagcgtcaacccgggcaccgactacgcgcagcgtcgcggcgtcgaggtcgtcgccatcgcctccggcacggtcacctggacggacaccaacccggacggctccggcggtcgcatgatcggcgtgaccttcgacaccggggcctacgccgagtacctgcacctgtcgacgatcagcgtccgcccgggcgctcgcgtcgagcaggggcaggccctcggcacgtccggcggatccgcgtacgggtccgaggcgggcgtcggcacgcacctgcacctgacgttccgcccgtacggccgggggaaggcgaacgccgacttcgaggacttcgtcggcggggcggacgctgcgcccgcgacgtcgggcgaggtcgggtggaagggcattcaggaaatgctcgcggccctctacggctacaccggcaagatcgacggcatccccgggtccgggacgtggtcggcgatgcagcgcttcctcgcccgcaactggggatacaccggccgcgtcgacgggaaggcgcagctcgccgggctgacctggaaggcgacgcagcgatggctcgccgcccggtacggctacgcgggccgcatcgacggcatccccgggtccggcacgacgcaggccctcgcacgggcgggcgcggcgaatgcgtcggcgtactgacgccctcgccgcggccgggctcatcgcgggcggcctcgtcctcttcgtgctcttcggcttgtgcgtgctcgcgccggtatcatggcatctagccgtgtggatccattaccacatcaatcactaaggaagcaaccatgaataagaccgtcatgttcatcacgttcgccgccctcgtcctcgtcgccttcgtcgggtcggtcgtgctgctcgtcgtccgccccgacgcctcggcgacgttcatcgggcaggtcgtgcagctcctcggcctcgtgaccgtcgccgccggtaccttcgcggggatcggcaagctcggcgggcaggtcgagcaggtccgttcgcagaccaacggcacgctctcgaagctgtcctccgagcgcgacgccgccctcgccgagctggcacgccgcgacgggaaggccgcggccgagctgatcgtgcccgagcccgggacgccgttcggcggcgagagcgccgacgccggtcggaccaactacgggcaggacagcccgccccgacaccgcatgtaagctggtcgtccggccccacgacggccgacgcagcacgaaggccccccggctagtagccgaggggccttcgtcatgtccgggggcctacaggcccggtaggggcgtgtcctcctcgccgggggcggacgggagccgggtcgacgagccgaagcgctgctgcgccgactgacgggtgatcccgagcgctccgccgatgcccgcccacgagacgccccggtcgcgctgacgctcgaccgcgtgccgcagcgccgcgtcgacctcggccgtcagctccgacagctctcgcagctcgtcctcgtcgcaccatgccacgcgcttgccagcggcccggatcatgcggcgaaccatcgctaggtagtcggtcgtctcaacgctcattaggtgccctctcggcctcgtcgtcggcccctcggccgttcgtcgattcagtgtaagggccgagttgacacccgcgcaacgtcaggcttaccctgacgctatgaacaacatcgacctcatccagtccgacttccgctccctcgtcgtcctcgccgtcctggtgtgggcgctgctcatcggcgtgctgctgcgcctgaacgcgaagatggacgccgcacgtagcattgagcgccccaccgtgcagccctgcacgctcgacaccgaccccgaggagaccgaccgatgatcgacctatccggcctgaccgacgaggagctgcgccgcctcgaagcgctgctcgacgccgaccccgacccgaccctgtccgccttcgacgcgaagctgcgcgaggccatcgaccgggcgcggctcgaccacgtccacgagtcccgggcgcgacgtcgagcatgacgaccgagcctcgcaacatcgggggcaccctcgtccggcggaagctcagcttcgagtccggcttcgtgcagatcccgaacgcctacatgcgcgacccccgaaccggcttcaaggcgaaggggatcctcgcgcatctcatgtcgcatcaggacggcttcgaggtcagcctgacgagcctcgccgacgtcagcgaccgcgacggcctgaccgccgtccggtccggcgtcgaggagctagaggcggccgggtacctccgccgagagtcgaagagcggcgtcggggcacccggcacgtacggcacccggtggatcctgaccgagcccgccgagcccctgttcggccccgcgagttcatcggataaccgcatgaaccgaccagggccttcgttcggaaaccgcacggacagttcatgcgaaaaccgcacgcataaagaacaccacctaagaacactcaatacaggtactagagacaacccactaggggctgcgcccgcagctccgacctatcccaagatcggatgcaccaatggacagcacacccgccatcgcgccggagaccgctattgcgccgtctgcgcagcccctctcgacgatgcttgacctcgccccgctcgaagcggtcgagtccgcccgcctcgcgccgtgcgctcgcccgcgccgaggacggcacgggtcgcgcgctgctgacggcgtgcatcacgatggaggccatcgccctgctcgtgcgggcaggcgactgtgatcccgtcatcgcggccgacttcgcggacgccgggctccgcctcgccgggtcgatccgctaggctccgaggctatgagtcgacaccacaagcgggcgggctggacgccgaaggttgcgcagcgccacgagcgccgcaaccgcgccagcctgcccgcgctgtgcgtgaacggctgcggtcggctcatcacgcctgacatgacgtacggcatcgactgggagaacggtcacttcgacaacctcgccgagggtggatcggtcaagctcacgggtccggctcacgtcaagtgcaaccgaggagcaggcggcaggctcggcgcatccatcaccaacggacgacgtcgagcacgcgatgccgaggacaagcagcagaccaacggactccgcccgtggtaacgaagcggatatccgagcagcggccgacgcaatcgacgtcgctcttcgaaatcgaaagcgaatcggacgcgaaggccgattcttttggtgtgctccgagacccccggttacccgtcagtcacccttttattttcgggggtcgggcagagcagccgggcgcagctccggccgggccgcagggcgctatcgcgtcg

SEQ ID NO: 2 - DNA, 16134 bp, unidentified
  source 1..16134: mol_type = genomic DNA
atggtgacgaagcgcaagagcgagctcatcccgacccagggactcagcctcttcgagatcgaggagccggccgacgagccggccccgttctttgagagtgctccgagacccccggtacccgtcagcacaccttttgttttcgggaaccgggcagcgcgggaatccggggtgtcggccggcgcgaaagtgacgccgatcctcgacgccccttcgctccggcacgagtcgatcgcgccgctccattgctcggccttcgaccgggccgaggagtggcacgacgagttccgcgtcggctgggcgagcatggcgacgatggactcccggaccgggaagccgatcgaggcgaagccgctctcttgggtgatcgccgatgcgatgaacgcgcacgacgagaacggcgacccgatcgccgacaccatggcgatctgcgtcccccgccgggcggcgaagacgacctcgatgctcgccgtcgccatgggccgctgcctcagccggcccggctacgtcgtgctcttcacggcccagaccggcacgaaggcgtccgctcggttccgtgatctcatccgcgcgctcgaacgggtcaactcgaacgaagcatcgaggggcttccggatcctcaagggggccgggaatcaggtgatcgagttcgccaacggctcgctcttcatggtcgtcccgcccaagggcgagagcttccgaggtgacgcgggcgacctgctcatcctcgacgaggcccaggagcacgaccccgaggtcagcgaggatctcctcggcgcgatcctgcccgtgatggacacccgccccggggcgcagctcatcgtggccggcaccgcgggcgagcatcggtccggcctcttctgggacaccctggaggagggccgtgccggcgtcgtcggtacgggcatcgtcgagttcggggccgacccggacaccccgctccacatggagggcgagccggtcgaggggaccgtcgcggatcccgaggtgtggctcggagctcaccccggcatcggcacgctgacgaccatggccgtcatgcacaagcggttcggcaagctgccgcgtccccagttcatgcgcgagtatctcggcctctggcctgaggactactcacagggtgcgatcagcaagaagatctgggacgacgccgaggtcggcttcgtcgagcgccccgagcacttcgccctggccttcgacatcgacccgatggggacggccggcgcgatcgtcgccgcttggcgcgacgcgaagggcacggcctatatcgagatcatcgaccaccagccgggcacctcgtggatgctcgcgaccggcctccgcctgacgaagaagtaccgagtcagcgtgggccacgacaccatcggcgcggcgctcgtcgaggccgagacctgggcgaaggccaggcccaagccgaggctccacccgatcagcctccgcgacgtgggggccggctgctcgacgttcatgcgcgacctcaccgacggcacgctcaagcacttcggccagcccggcatgaccgacgcggcgctcggatccgcgaagcgcccgctcctcggcgagaaggcgtgggcgtggggccgggccgcgagctcgtcggatatcacgcctctgatcgccgcgacccatgcgctccgcgtgtacgatacggcggagcgccggtccggcgtcggactcatcacagcgaaggcgggataggcattgggaatcagaagcgcatggagggccagtcaggcgatcggcaccggggcgatcgtctccccgtggtcggagggtgacctcgccaagatcgtctggagcgacgtgctcgggacgacgccgtcggtcatcacgcgcgccgaggcgatgaccctctcggccgtcgtcaaggcccggtcgatcctggtcgggcagatcgcccgctggcctctcgtcatgctcgcgtcggactcggccgagaaggacgcgactcagccgaagtggctccagtccaccgacggcgagatctcgccgtggcaccggatgatgctgacggtcgatgaccacatcttctacggctatgccctgtggctcgtcgagcgcgacggcacgggcgagatccagcgggccgagcacgtggctcagtccgagtggcgcttcgaccaggacggcgcgatcgtcatccgcgacaccgtcgtccccgaggccaagtgcatcctcatccccggccccttcgaggggctcctcacgctcgccacccgcacggtccgcggcgggatctcgatggagaaggcctgggtcggcaaggcccagaaccccgtgcccgtgctcgacctccaccgcgactcggacgacatgacccaggaggaggtggaagacatgatccagggctgggtggacgcacgtgccagcgagaacgggatgatcagctcgacccccgccggggtcactccctcggccctgggcgagaccgacccgcagctctacgtggagggacgcaacgccttccgcctcgacgtggccggcttcctcgcgatccccggctcgatcatggacgcctcgaccgccacggcctccctcacctacgtgacccaggagggcaagcgatccgagttcgcggacatgacgctcccctactggatggaccccatcgcggcgcgcctctcgatggacgatgtcgtcccgtcgggcagccgtgtacgcttcgacctcagcgacgcattcgctgtgacgccggcacccgccggaccgaccacgagagactaggaacccatgaccgtagtcaagatccaggcgggtacgatgaccgcctcgctggaggaccggaccgtgtccggcatcctcctcccgttcggggaggtggggcggacgaacgtcggccgcatcatgttcgcgtccgggaccgtcgaggttcccgaggacctgagcatcgtcctcggcaacaccgaccacgaccgggagaaccccgtcgccacggccacgcacatcagcgagaccgaggccggcatgttctcgatcttccggatcgcgaagaccccggagggtgactcgctcctcgccgagatcgcagacaaggcgaaccccgacgcccgacggatgctctccgccgaggtcaaggggatcacgaccgactcgaaggggaaggccctctcgggcaagctcttcggcgcggcgttcgtcaagtccggcgcgttcccgtctgcgaccctcttcgctgccgacttcggcggcgaggcagagggcgaggagaccggcaccggcctcacgcccaacgacgagggcaccatcaccatccaggccaccgcctacccggaggccgtcgaggtcgccggccccgccgaggacggcgcgcccgcgtcgatcctctacaccccgagcacgatcgcagaagaaggatcctccacgaccatgaccgcccaccgcgtccacggacagaccacgaagaccgacgagaagggcctcggcctgaccggcttcttccagctcatggcagaggcgtaccgcacccggaaccacgacctcctcgcccgggtccacgaggagagcgtcgcggggaacacgatgttcgccgcgctccaggacgtgaagagctcgggcgcgaccgcgaacggcggcgcaccgaacgcctggcagcggccccagtggctcggcgagctctgggagggcaaggccttcgagcgtcggatcatcccgctcttcggtcacgccgacctcggggcgctggagatgagcggctggaagtgggagaagaagccgacgatgggcaagtgggccggcgacaagacgccgatcccgtccgacaccgtcaagacgaagacggtcaagaaggaggccgaccggtacgccggcggccatgacatcgcccgcgagctccgcgacttcccgaaccccgagttctgggagggctacttcaaggccatgaccgagagctacgcgaagctctccgatcagggcgtctgggaggacgtgctcgctgaggcccagtacctccagcccggcgcggtcccggccggcgtctcgtccggcatgacgaagatcgtggacggcgcgatctccatggtcgacttcgcgctcccgtcgttcgcggtcgtcgcgaaggacgtctaccgcgaggtcctcctcacccgcaacgacgacacgctcgcctacctgaacgcgtccctcgggctggaggagggcacggtgaccaacttcaaggtcatcccccaggcgatgccggccggcaccgtcctcgtcggctcctcgtcggctgccacggtccacgagctccccggatccccgatccggaccgaggcgctggacatgatcaagggcggcatcgatgaggcgctcttcgggtacgcgggcgtcatggtccacgacgtgcgcgcgctgaccctcgtcggcgcgacccaggcctcggccgacccccgctagctcgtcccctcgccggccggccccacctcggggccggccggccctcttgctctcggaaggagcgcccgtcatggggtacgtcaagcaagtctggaagaacctgagggccggcaacacgccgctctcggcgaaccgcctgaaccacatggaggacggcatcgaggaggcatcgctcgcgggcgaccgtctcggcacccgcgtcacgaagctagaggcgggggccggcacgaccgacccgacgaaccccgccccgacctggacggtcgccaagtccgccgacccggccggcaccctcgtgccctactcgtcgtccgccttcctcttcaccggcaacggcccgaccgcctccggtcgctactaccgcaacaccgtccagacgaacacgcactcctccttcgagttcgtcacgtcctccgatgtcatctacatccccctggtcggagtccagaccatcggctcggtctacgcggacgacgtgctcgtcaacgtcggcgaggacattcggaccgactcgtccggcgcggcctacatcctgaccgtgaacttcggctcgaagaagtcgcgccgcatcaagtggaccgcggtgaaccagggcttcggcggcgtcatcgtcccggccggcaacaccgtcacggccccgagcccgaaggccaagccggcctggggcctcggcgactcctacatgttcggcgtcggggccaagccgatcagcgagtcgagcttcaccgtcatgtgccgcgagctcgggtgggacggcctcgctgacggcatcggcggctccggcttcatcacggcctcgccggacgcgaacggcgtgatcgccttcacgaaccccgccgaccggatggacaagaagctcaagaccctcacccgcctgagctcgctcctctacggcgtcctggacctcgggctcaacaacgccgcgagctcgctcgacgacgtgctcgccggcttcgacgcggcgatcgccaagtgggagaccacggccccgagcgcggcccgcctcttcgtcatcggcccggcgttcccccgtggcgcgacgacggcgctgacggcgatggatgcggcgttcgctgcccggtgcaagaagctcgggtatgactacgtcagtcaggccggctggatcacgagcgccaacatggagctctacaccatgcagaccgagacgccgcccacgcacccgacgccggccggccacgagtacctgggcaagcggaaggcgacggcgatcgccgcgctcatcgccgccgactccgacggccccgaccctgagctcgctctccacgaccccgggatctcgaaccccgatcaccgctacgtcgcgagccggctcggcctgggcaccggtgccaccctcacccggtggcccgacctcggcacgaaccccgccgacctcatccccggcacggccgcgtccggctcggtcggctcggcgaagtacgtctcggacgccgatgggggctacgtccgcctcgtctccgcgtcgggcaacgccttcaccctcgcgaccgtcgccctcgtcggcacggcccgcacgacgaccctcgtcgtccgcgcggcaaaggcccggcagatcctccggaacgcgggcgcgctgctcgcccgcgcctcgagtggatcgttcaccctgaccgcctccggcaccggctccggcggccagctcctcatctcgaccgccgtcagcaccgacgagtggaccgtgatcacggtggccgccgcgccgaccggggccgtcctcttcgtcaacggcatcaagtgggtgagcgccacgtggacggccggcgcggagacgaacctccgcctcatggcttccgaagcggaagacggcccgaccgacttccgcgaggtcgtcagcgtccagcgggtcgtcaccgagaccgaggccctctcgatgtataccgccatgcagacccagtacgcatccgtctagggagaacaccatgtcactcgtcaccaccgccgagaacctcggcacctactgggccggcgaccgcccgccctcgctcctcttcatcgacctctccggcgacaacggcgaggaggtccagctccagggcttcgagctctcggcccgcctgtaccacaccgagacgatgttcctgtcggtcccgctcacgatcgaccccttcgaggagaccgactccccgggcggcccggccgtcggcgagacggcccccggccgcgtcgtcgtcacctggcccgacgaaagcatcctccaggagcccggcgtctatgagatcgtcatcacgctccgctccgaggacggccgcatcctcctgaccggcgacgccctccgcttcgtcgtccaggcgcgcgacgggtgggccgacctcggccgagctcggcacgactgggccgacgcccccgagtccgacgtgaccctcttcgagatgctccgggtcgcccgagctcaggtcctggagtacgcgccggccctgccctacggcacccgggtcccggtcaactacgtccaggcccaggtactccaggcccgggccctcgcccgcctcaacgccgagagcccctccggcctcggccccgacgggaacgtgatccagatctacccgctggactggaacatcaagcaaacgctccggccccagaacccccgaccggtcctcggatgaccgtccggacccgactcatcgccgagctcacggcggcgctcgacgcccagaggttcgtggtgaagaagtcggcgaagacccccgaccgcctggagaggagcaaggcgacgctcctcgtgcagcgtgatagcttcgccccgtggaataccccgaagtcgatgcgtcacgagttcaccctcgcgctgctcgacgcccaggagatcgacgccgacgaagacctcgaagactcgacggacgagcttgtcgccgtgctcgacgggatgggggagctctactggacggcggctgaaagggcagtattcgacgacaagtggcattgttatctcatcaaggtttcactcatcaccacatataaggagaaataagaaatggcaaacaccgagccggcgaagttccagccgctattcctgcgcgactattccgtcatcgtgcgcggcgtcgcggacggaaaggactacgcccgtcagattagctccatcacgatgacgccgacctcggccgcatccacctggaagggcggcaaggagaacgcgagctacaccgcccaggcgtcccccgactggacggccgcgatcgagtccgcccaggactgggagaaccccgacagcttctccaacttctgcttcgccaaccagggcaaggaggtcgatgcatccttcgtccccacctccgggcagggcgtcgtctgggacttccgcgcgatcgtcgcggccggccccatcggcggcggcgtcggcgctcacgcggcggcctcggtctcctggggcctccagggtggcccgaagccgcgcgcgtacgcggcggcgaaggacgccgtcccggcaccggcctaggcgatgatctccgctaagcggtcgcccgagctccaggcgacgatcttccggctcaagaccgtgaacgcggagctccgcaagaccctgtatcgcgcggcccgtcagactctccggcaagcctggaccgaagagctggcgggtcgcgcgtcctcgtccctacaggagcgcgtcctagtcggcggcgctcgaacggtcgtctcgacccagggcttcaaggtcacgacggcgaagcaaacccgcgccctctcgggtggcttcgtcccggcgaaggactggccggctgccgagttcggcgcaaagtggcggcgggcgaagatccgcagcacctccaccctcggcaaggccttcaccgtgagcaaggtaatcaataagcaactcaagccgagaaaccggaaaggctacgtcgctatgccttccgctaatgatatcggcattcgtctcgtctccctttgggtccaagtaatcgcgcgcgaataccacaacgcgtcggaaggtaagtaaatggctggcaagggaatcgagttcaccttcatatccgaaacacgggatatgatccgtgggacaaaggatatcgagaaggctctcgaaaacgtccaggattcagtggacgacgttgccaaggccggcgaggggttcgatgccggcgacgcgatggcggccgacatgaaagccggcggagccaagtcggagaccgctctcgatcgcctcatggacaagctccgcttgaccgagaagaagggcaagatcggtcgcggcatgggcgacgagatcggcgacgggatcaagaagggaaccaagcgcggcgaggagggcctccaggagttccgcgacgaggccaactcgaccgcgaaggagagcgccgcctccttcgacggatccttcgagtcggctctcgactcggtccaggagatcctggcaaacgccctcgccggcttcggccccatgggcgcggtcgccggcctcgctctcgcggccggcctcggcgcggcgatcaccgccggccaggacgccgccgatgccgtcaacgaaacgaagacccggatcggcgagctcgccgaggaggtcgtcgccgcgggcggtgatatctcccaggtggacctggcctcgcggatgcgcgagtggggcgtcgagatccaggatcagcgcgagctgtgggagctctggcaggactccgcgaagtcgaacatcgaccatgcggccgacgccgcgaagaccgccggcaccgacttcaagaccatgttccgggccctgtccggtcaggacgcgggcgcgaaccagcgcgccctatccacggtcaactcccagattgaggatctggaggacaagatccgttcggctcgcgccgcgggcaacctcttcgccggcctccaggacaccgacgggatcgcgctcaactccctccgcggcgtgcgccgtgagctcaccggagtgaaggacgagcggaccgccgcgcagaaggccgccgagctcctccaggaagcgaccgaggaggagaccgcagcggcccaggcgaacgccgacgccgaggccgcagcggcgcgcgcgaccgagtcccgcgcggccatggcctccgccctccagtcgggcctggacggggccgtctccagctactccgagttcaccgacgccgagaagggcacgaccgatccggggaagtacgtcgccgccatgcgcgagcgcatcgaggcgacctccggcttctcgtctcgggtcgccaacctcgcgaccgagttcggcctcagccaagctgagacccaggcgatcctggatcagggcgtcgagttcggcccgatgctcaagagcatccaggactccggcctctcgggcgagttcgtcgcccagatccgcaaggccgtcggcgggggccaggagctcctggacggcaccgagctcggcacgaccgtggacgtggatgccgacccctcgaaggcggagggcaagctcgacgcgacccaggggaagaagcgcgacgcgaagatcgacgccgacgccgacaccggggccgcggcgaaggagctcgaccagaccgccgcgaaggcgcgcgtcgcccggatcctcgcccaggcggacgtgggcctcgcgtccttcctgctcggcgtcacggccgccgtgccccgctcggctaggatcacggccgtagcctcgaccggccaggcgaacgccgacctcgacgccctggcctcgcgtcgccggacgacgaccatcgtcgcccgggtagtagaccgcaccggtaaggaagtgaactagtggcaacgatcacgtacgggacgacggtcctccgaccccgtctcgtcatctcgcacgcgacggcccgcgtctcgccgaacatcgtccacccgatcctcggtcgcgccgcaccgtcggtcacgacccggccggcgcagctcaggaccgggaccctggaggtcctcttcgacgacgagtgggaagccttcgccgcggagaacgtgctcgcgacgccgggcatcttcgccctggaggacgggtccgatccgacctacggcatggagttcgccgtccagggcgagatccgacgcaccctcgacgaggccaccggcaaggcgtggatcctctcggtcggcttcgtcgaggtccgcctcccggtcgatccccgctacccggcggccgacctctacccgtccgaggagcgcatccccgcatgagcgtccagatgcacaccgtcgaggcggccgtcctcggcccggtccggatcccgctcgcgatccaggaggccaccctcacgatggacgagggatggtcgcccttcatccaggccgacctgacgtgccggctggatgacgttgccgccgcctacaccatcgacccgaccttgcagcccctccgggtgtcgctgaccatgtccgcccgctcggccgccggcttgcctctcgcgctgctctcggcggccttcgccgggggccggctctcggacctctcggaggcgtacgcgaacgcggccgttagcgacgtgtcggccgactactcggtcccggggcagcggctcgacgacgacccgccggcctcgcggatccaggtgaacctgtcgctccgagctcgggagatcgacctagagaccgggacgatgctgctccgctgctcgtccgacgaggccctcctccaggacttcggtcatgccgtccgcgatgcctacgccggcaactcgacccaggtccgcacgcacgtccagttcgtcctgggccggctcggcttcgtgctcgaaccggacaccctcgacgatgcaccgatggaccccgaggcggcggtctgggatcccggggtggatgcctggtcgcacgtctccggaccggtctcgaaggccgacctccggctatggtgcgacggcgatcgccggtggcacctgacgaaggccggccccgatcgacccggcgacggccaggacctcctggcccagttcgccgtgaccgccggccaggacgccgtcagcatggacgccgactggttcgacgccgtcgtcatccgctaccgatggtccgaggacaacgccgacggcggctccgagtccttcgtcaggtacgacaccgcgacgatgcccggataccggaaggtcaagacgatcgacctggagacccgcttcccggggtacggtgccgcgatcgcgatccttcgccggaagtggcgcaagagccgagaggtcccgacgaccctcgtcagccactacggcgcgaccccgaaccgcctcgtcgcgatcgcgcggccggcccctcacccgatcgtcctcggtcgggtcacgtccgtatcctgggcgttccccgccgacgagatgatcgtcaagacccgagtagagaagtgagaccatgaccgcaggatccggatacatcgacccccagaccggggtctacatctacggcgaggacgacctcgtcggcacggagttctccgagctcctcaacctcgggcagcgggcgatgggcaccgtcgtcaccggcctggagaagggccggatcctcggcagctacgacgccccgtgggtcggcggcggctttcggtggcgcgaacggtacgcccgcctgtactcgtggacgatcccggatccgggcgtcccgtaccgcgtccagatcgaggccggcgccgagatcggcaccgagtccggatcgacccgagctcgctacgacatgcacatcggcctccagcaagccggcggccagtaccggcagatcggcggggcgatcaactcgacggcggagttcatctaccagaactacacctcggccccgctgccccaggtcctcgccggctcgtgggacgtggtcgtcatggcctaccgcgtgttccccgaggctgatacggacggcctctggggcgagatcacgggcgtgaaccgcctactccgcatcgtcacctactcggcctgagcgttaggatgcccgcatgagcacatacattcaccccgcatcaaccgagctcgggatctccgacgacttcgccgcgcacgtccgccggcactcggtcaaccccggcaccgactaccgcctccgcttcggctcgcccgtcgtggcgatcgccgacgggaaggtcgccttcatcgacaacgtccccgatgggtccggcggtcgcatggtcggcatcaaccactcgaacggctcctacaccgagtcactccacctctcctcgatcgccgtcaagaagggccaggccgtcacccagggccaggagatcggcaagtccggcgcgtcggccaacggcaaggagtacggcgtcggcacgcacctccacctgaccttccgcccgcgcggggtcaaggacctgaacgcggacttcgaggtctgggtcaaggccggcgaggtggacggcggcgtcatcgttccgagctcgccctccggctcgtgggtcggcatccagaagatgctggcgaagctctacgggtacgaaggggagatcgacaacgtcgccggggcgggcacgatcgccgccttccagcggttcctgacgaaggtctggggctaccgcggcccgatcgacggcgtcgcctcgaagggcggcaacacctggaaggcggcccagcggtggctggccgcgcgctacggctaccgcggccttatcgacgggatccccggggacggcaccatggccgctctcgctcgggcgtccgaggccaatgcctcggccttctgagctgctcgtgacgggcggcctcctcctcctcggggcggccgccttcgtcgcgtatgggctctacgtcctcccgcgcgtcgcgatcgcgctcctcttcggctccctcgtcctcatctactcgcactaaggaaactcacagcatgaacaaaacgaccatgttcctggccttcgtggccctcgccgccctcggcctcatcggcacggcggtcctcctcgtgctccggcccgaggcggtcggcaccctgaccgcgctcctgacgcagatcctcggcctcgcggtcacggcggccgtgaccttctacggcctcggtcaagtgaaggagggcatcgagaccgtgcgcaagcaaggcaacgggacgctctcgaagctcctcgccgagcgcgacgccgcgacgaccgctctcgcgatccacgcgccggacgtggcctcgaccctcgtcgccgcccgcaccggatccgacccgaccctcgacgtggttgacaggcagggccggcacgaggcagagtaggcctcgcgaccggccatggttgctcctaccgggaacgcccctcagtccatcgggaccgaggggcgttcctatgtccagggctcggtccgcatcgcctcgaaggccgagaagggcacgcggccatgctcgcggaaccactcgcgcagctcgtccgaggcgtaggcgttggcgcgcacggcgttgcccatgaagagggatcgcgactcgatgcccgcccgccggccccggtcattcaggagcgcgcctcgacagtcctcggcggcccgagagtaggtcgcttcgaggtagtcctcatactcggcgcggagctcgcgccacctctcgacgccggccgcgatcgaggggctactcattgactgcccagtcgaggatcacgacctcgacctcgccctcctcctcggtgggcgcttcggcgtaccgcttccaggcggcctggtgcgagatgcccagcgcctcgcccagagctcgccacgagcggcccgtggcgcgctgcccctggaccgcctgggtgatcgcctcatcgagcacctcgcgcagcttcccgagctcggcgagctcgacctcgtcggcgtccgccacgcgccggccagcggcccggatgaaccgtcgggcggctcctaggtagtccatggtctccacgctcatctgagctcctctgttagtcccggccggcggctcggggttcgtcgatctgtagtcaacgtagcttgacaagctcgctcccgtcaatctaggttgaagccatgacgaacacatacagcaacaccgagctccgttacctcatcccggtcctgaccctcgtggaccgcggccacggccaccacttccgcccgaccgtcctcgaccgcctcgaagtcgccggcctcatcgagcgccccggcttcggcttcgtcgtcctgaccgaggcgggcaaggccgtcatcaagggcggcccccacggcttcacggtggccgcctgatgatcgacgagatccccatggtgcccggcctcatcgtggccctcgtgctctgggtcatctacctcctcgcccgcaaggtcatccgggacgaccagacgccccacccggacgactactctcaagacctcaacctctcccacctcgaccgtaaggacggcctccagtgatccgcttgaccatcgacctcgacccgaccgaggaggaggccctccgccgccaactccagcagatcgcccattactcggacctgttggccgaccgcgccgtgtccgagcggatcctccgcgagctcagcgtctcgaccgcgcacgactggagccggcccaaggcggagccggcgtggggagagctcaaggtcgccaagttcaacccgtggccggcggcgctcctcgcgggggtcggtgcggtcgtcggcaccttcgtgggcgtcgtgggcctctgggccttcgccggcctcgtgtagtgcagatccggatagtcgagcaccccctcacgcccgccctgctcgtccacgtggacgagtacgggcgggcgacgtactcgacgaacaagctcgacagtcaggtcgtcaacctcctgcgcgcccttgcggaccagatcgaggaccagatccccatggccgcccgatgagcgtcgagagcctcgcgatcgtgctccatcactcgcgagcgaagggcgcggccaaggtgatcatgctcggcatcgccaaccacgacggcgacggcggggcatggccctcgctgacgaccctcgcgaagtacgcgaacgtcaaccgagaccaggcccgcaagctcgtcgccgacctcgaacgccgaggcgaggtgcgccgcgtcgtgaacggcgggggccggctcgacaccccggactacctccggccgaacctctaccagatgctcgtgcgctgcccgcctgactgcgaccggtcgcctcagcatcggaccccgaaggaccgcgaggccgtcacgttcatccccggcctggagccgctcgacgagaccccccctcctcagtcacccccggtcacagaggaggggggccccgggtcaccgacgacgggaggggggggtcacacagacccccctaaccgtcctactaaccaaccacctagagatccagagaagaagccggcttatcgcgtgtgcgcgcacgcgaggccacgaggaggcccgcatgtctacatcagctcaccgaggtactgcgaacgatgcggatacgaccaggaggtccatggactctctagctgagtccgaggccgcatgctggcgggcgggcgacgtggacgccgccctccagctcgcggcactagaggtcagctaccaggccggcggggtgtccgagctcatgcttgcgtcgtgggccgaggcggcccgcctctaccgccctcgtgtaccatcccgaccatgagcaagcaccacaaggcggcagggtggaactaccgcctcagccagacgcacagcaagcgcaaccgcgccacgctgcccgccttgtgcatccagggatgcggccggatgatcacgcctgatctccagtacggcaaggactgggagaacggacacctcgtggatctctcggccggcggcaacgtgaaccgcaccggccccgcccatgtgaagtgcaaccgtgccgcgggtggcaagcgaggtgccgccctcacgaacggcacccgtcgagccgaggcgaaggacgacaagaagctccgtcc